European Patent Application EP 4 298 896 A1, published January 3, 2024. Title: NOVEL QTLS CONFERRING RESISTANCE TO CUCUMBER MOSAIC VIRUS. Applicant: Seminis Vegetable Seeds, Inc. The sequence listing filed with the application follows.

SEQUENCE LISTING (35 sequences)

SEQ ID NO: 1 - DNA, 2000 bp, Cucumis sativus
  source 1..2000: mol_type = genomic DNA
aaatcaggattagactctccataaaaacaataagaaagaaataaatggaaggaagtagacagactccgcagtccgtacgagaaaaaacgctgtgaacgccctcctcatttcgctacctctttccccttaactttgagtatttcacaagtcatccttccttttctttcctatttcttttcttcacgtcatcctcttttttctttctttcttaattatttaatttcacaaccatcatttgaaaatataaatatatatgtagctaaattacatatttagtcttctcaacaatctcaactcttaaaatggtaaaaataggctaattatataagaaaatactctataatattctcatttattcctttctaaaaatgggaattgctattttttttttccttccaaaagttgtaaattgtaatactacatttgattgattgttttcaaggttgtcttataagttggacgaaaattgaaattagaaaatagtataagtaaatatggaggggtgtactgactatttttgaaatcattgaaaatctctcaaataactcaccacaataattttttctctatcacattcactactctacctcaagaatgaaattaaaatttaactaatgtttcatcatatatccaaactataagttgttttaacattcaattttagaaaatattaaatgagatttttaaaaatttgtagcaaactaaaaaaaaagggtattttagacaatatttcatatatataaatacatatattccataatgcatttgcttgtctgtgggagtggtgtggtatttgcattatattaaaaaccagtggagtttgtttgatttaggagttgtgtatagtgagagaagagagcagagagcagagtgaagaaagaaaagcaatggcgagtttggaacgaacccccacatgggcagtggccactgtctgctttttgttgattctcatttccatttccacagaatatttgcttcactttcttgtcaaacgggtactgtactaccccaacaaccaaatttcttcttcttcttcttcttcttctttcttcacattatttcattttcagtttttcagcatcaaaagaaggaaatccctcaggcaagctctcgacaatatcaaatccggtgcgctctctcaattcaatagtatatttattattactagccaactatttaattgattatcttaattctaaagaaaaaattatgtggtggatatgtttgtgtatatatttctacagaattgatgcttttgggatttgtatcgctgttattgacggtgagcgagaaaggaattgctaacatttgcattcctaagagtttgaatcacaaatttctgccctgtcacactatcaacttcaattccacttacttcttggaagaacccaagtgtgattcacaggtaaattaactaaaactaaaattcatacacgaacacaaaaacattattataatatatatatatatatattgttaatttgaaattatacttcgctgtttaatttggtaatttgcaggggaaagcttcattgctgtctagagatggtgcaaagcaagttaagtatttgatcatttgtttagcctttgttcatatcttctccagtctactcagctatagtcttggaatcgccaaggtacctattttcctttcctctaatacaaacataattcaattaacttagacattgaataaaagaaaagaagaaaaaaaaatggatataaaagtcattgaagaagatgtgaaagaaaatatggttgatgtgatgatagacttgaccaaatgtgaaggttatgcgtagtttagagtagctgtgtagggtaatgataagaattttacataaatttatttggggcaagacttttgagatgcgtacacataaaacttcactatcctcaataatatttgttcgttaaatcctctgtctacttcttcaaattccattttattggactaattacatacttttttcaatttatttactgcactccatgccaac

SEQ ID NO: 2 - DNA, 200 bp, Cucumis sativus
  source 1..200: mol_type = genomic DNA
agagtatggacaccaaattctgttacttcaacaattacaatgttaatcagcctagacatttctgcaagggttgtcaaaggtactggacggccggtggggcgctccgtaacgtacccatcggagctggtcgtcgaagagccaagccgccgcctaattgccggaccctttccggcgagctgtctgaggattatgggcagtat

SEQ ID NO: 3 - DNA, 200 bp, Cucumis sativus
  source 1..200: mol_type = genomic DNA
cattttgagttatactttacatattgaactgatagtttcgtttttgcaaactcaatccaacgttacattgcttatgtatgcctctaatatattagaaacaaaatcggcatgaattaaaaaaaatgcaacctttacaaaataagagacctaaataatttatcaaacaaaacccaagtaagaacctaattgaaaaggttaat

SEQ ID NO: 4 - DNA, 200 bp, Cucumis sativus
  source 1..200: mol_type = genomic DNA
tcaacctctcaggaagatggttcaaaattgtctgtcctgaacgctgaatgtatggacttaaggaatagagtagagcacttgcaagttttgctagacaaggcaaccgagcaggcagatcaagctattcgtgttttgcaacaaaaccaagagcttcaagaaaaggttgagaaattggaagagtctcttgaagaagctaacgc

SEQ ID NO: 5 - DNA, 200 bp, Cucumis sativus
  source 1..200: mol_type = genomic DNA
tggtttgtttatttaatttttttcttcttatggctgacatccaagtatatattgcagtttcaggaaaatacaaaactacccaccacgtatgcctttgcattagtggaaagtcgccaacaaagtaaactcaggcttcgaatgtatttggcgggagaagtcacacataaagacgtagaggcaatcgtatcttctccaagact

SEQ ID NO: 6 - DNA, 200 bp, Cucumis sativus
  source 1..200: mol_type = genomic DNA
caagaaaactgaaaggaatcaacttcatgatcaccaatgagttgacagcaataaaagggcaatgggcaatgtgtgtgtgtttttcttcattgtaggcaaactgctttcattgagaaaaaattaaaaagagcaacgtttgtatgtagataagacctatattatattacaaagaaccaagttttcattgagaaaaaaatgga

SEQ ID NO: 7 - DNA, 200 bp, Cucumis sativus
  source 1..200: mol_type = genomic DNA
tgagtctgaattttttgtaaaccctaggggtgggtgagggagggaagctaagggggggagggggggctagggtttgtaattcatacagaggtggaggatcttttttctctggaattgcagctgtttttaagatttttgtatttgcaggcagccgttgtaagattttgttgtttagggatggagactagaccttatcattt

SEQ ID NO: 8 - DNA, 200 bp, Cucumis sativus
  source 1..200: mol_type = genomic DNA
ttcatcctgagttattttaaaaccttttaaaaatttaagacttgtatcttttataattttaatcttaaatagaaagtagttttagaattataattctttttttttctatattttataataatttcaatatttatttttaaaaaataaataaatatgcaatattatgtataaataaagaaggaaagtaggggggagacgta

SEQ ID NO: 9 - DNA, 200 bp, Cucumis sativus
  source 1..200: mol_type = genomic DNA
agatgaaaataaatcacacaggatttaattgatttctgtaaagaaacgggtcttcagtccagtgctgcggctacaaggaatgttactattaagcttttgggttgcgtgcataaatttgttggaccaggtgactggatccattctttctgtttcttggaccataacttgaatccttgataatataattcctcttctctaac

SEQ ID NO: 10 - DNA, 2000 bp, Cucumis sativus
  source 1..2000: mol_type = genomic DNA
agaaacatgaacaatagtatttatctagaatagtactccttccatgaaatttctatgatatatggcagacattctcaccttgagtggtttagacttgtcataccgccctcctgcaggattagcagcagcgaggattgatgtcctagcatttagtgtggcctgtattccggcttttgttatgcttatggtctgctgctccatagcttcatgaattgcaaccttcaatagcatttgcaagccaaattgatcaagaaaaggcatgagatgcagcattaaagcattgacaaaatatatagcaagttacctgatccctgatgtccattttgtcaaattcatcaatacagcaaataccattgtcggcaagcatcaaggcaccagcctgcaattaaattagaaagaatcaagggaactacagaaattatttcacttcaatcaatggttatatgcattagttggcagtttatgctaagagtcctataagcactatgtatgcatccaacaagatgagacagattttagtaaaaataactttttattagaactatgaagtgggatgagatgaatcttaaacttgacattaggaaaatttctctcctgtttctagtcagcctattaagggtaccaccatctgaccaaaaattacaaaatactaaggtacctgtgtagatgatgaatatcaaataaaatgctacctcaatacaaaattccccagtttctggttctttggctacagttgcagtcaatccagcagcagaagaggactttccagatgtgtaaactgatcttggcacaatacctgaagtatacctgcagaaagcagtcatgaattaaggtctgtttgataaacttcttgaatggaaaaagacatgcaatataatgtgtggagaactagccagctgattggttaaatgttgacttcagagaaatggaggaaaaaataatggtaataataaataaataaaaatgctagaaactgaacaaggatttgtatagtgacaaatgggcaagcaatgaactaagatgtctattagggcatggatttataatcaaacaagctttctcgatattaaatgttatggatcaacagtattatgtgtatgtttttaagcataaggtgcaatattaagcacaataatctttagaggtcttggagcgaaaaaagagtaaaggttattcttcaatgcatacaccacgcaatgtaatacaaaaaactaaagaaagacatgcatacgtatatacgggtttttaagaaatctttccatttaaagggaaaaaaagcttaaatattgcaagtatgtgtgtggtgtgccatgtggtggcgtgaggtccccatggctctttcgttcttcacttttttaagcaatgacactgtgtgggataagtgaacatccacagccgtaaatcataaaaccctgaactattggctgtaaaagctccactttatggatggacttttcacttagttcaaacatcaaaaagccaaacagaaatttctgaagcaccatttactttggaaaaagcatacctcctgccgcattcaaaactctacagagttgttgagaagttcaaagtttaaactaagaaccagaacggaataaggaaaaatataaaaacttacttaagaaactgagatttcgcacagcttggatctcctactatacagacgttgatgtcacctcgaaggttaatgccttcatgagttaacttgtggacaccacctaacagcatcagcaagattgctcgcttgatgtcttgatggccaaagactgcaggtgcaatgctatcaacaagtctgttgaaaaagtcaggtgtattcctcatcctttgaacgtcatccagctctccagtctgaagattttgttatctaaatctaagtttagaaattcttggccagcatatgctggagaattttaaaacgtttaagcttttatttatagaagacttgttacaaactaactagtaaaatagaataccacaatgattacctagaagcttaatag

SEQ ID NO: 11 - DNA, 2000 bp, Cucumis sativus
  source 1..2000: mol_type = genomic DNA
ccttggagtcaacgggtgtcaattgagctaacattttgttgacacaattttaattattaagaaccgttagatataggtctaccctccgtagacataggcctatcaatacactaataaacataggcctatcaaccatacttactattagatgtaggcttatcaacgatggacatgtttgggaaaggtttatggaggattagagttatcataatacctcaattcttgtttaggggagggttatcataatctcctataacactcctttgtctttattttcgaattttcacaactctattattcttgtattagtgaaattttgtaaagattaaaaaatatatataattttatttttccttataaaagtattaaaattttagttttagtttttttaactcgatattgtattttaaaatattagtagtaggtggacgctaaactttaaaaaaaagaaacttatgaaaactaattttataaggttattttttaaaaaaaagcagaaagtataatattttgaccgtttcgtacgaataatcatttggtttttatttttgtttcttttataaaaatttagcttacgaacacttttttattaactagttatatttttttaatgtatatccaataaataaatttaatatatttgttttaataaattaggaagtaatttcagttataaaaaattatttttttttaaaaaaaaattcttctagatcctttagttttcttgtgctttaaaaaatcagccttcatttagtaactttatgttttctatttcttattaaaataatctttttacatttttttataatatttgttaaatctagtatgtcattgctatactttatttttctaatgtactgtatcaatagaatttaaaatggtgttagttgtgaaaaatagaaaaattatttttaaatggttagaatagcttaacagaaacaaaaaatagatagaacaatgcctcaaatgctctaccaattgaaatccctagaactcaaatatgttacaggtctatattcgtggacacagaaagcttttggtatcatctcaaaatgcctcattccaatggagatagttgtccttacttatatacccaacatcattctcttataaccgataagggactttggtcagattcacaatccttcccttgaacaatttccatattacaatcctcccctcaaacaaattacctcctccccttaaatagtcatcccatccgtcaagctttatctaagctatctcctcttctcggagcaccctgtccatccgatagcaattacggatctcatcgtgactacttttgaggctttcgaggttctactacatctttgttcgacacctgtacatcatactagcatagtttggttaagttagaagcatgactttgataccagttgtctttcagaaaacatatctaaatttaaacttttgcttttagaagattataatatatctctataaagattactctcttaagcgtactactttattgtaatgatgagtgttacaaaatactggtcgttaaaatctcttcaattgtatattgtatgtgaataagtattcagtcgaattaatccggatatctttaaataatgggaagagattttctcagccttagataaaattattggtgaaattctcatttcatatagaaatacactgtaatttaaacatttgaaacatggtagaatttatctgtgtatatatgcacataaagattcctaccagacaatgcaatgcatgcatgagaacacatgatcatatgtaggtttcgttgccgacatgagcaagtatgatctagaatattgacaataaattgttcactaaagtggtgaacttcaaattcacgttggttcataagatttatgtgcaaaaggacattaaaataaatggtagatataaataagactcttaataatgataaccttaattattccaagaaacaaaaacttacatttgttgcacgactcttccttaatgctattcgaatcatatcc

SEQ ID NO: 12 - DNA, 200 bp, Cucumis sativus
  source 1..200: mol_type = genomic DNA
gtcgaaagatatccaaaatttgaatttagaatggtatcttcccctaaaatcatgcatttgatataacaacttcatattaaatttgttatttctcctatagttatgcatttaacgatgattttcataaaattgttcatttaacataataataaattgaaattaaaacttccataaaatggttcatttaacaatcattccat

SEQ ID NO: 13 - DNA, 200 bp, Cucumis sativus
  source 1..200: mol_type = genomic DNA
ttgctattttccaaactccactatattatttttccattctaacaaatttctcttttgcaaatgccccataaactaacttgttggagattgtattatatcaatctaaattattaatcaacaaaattcagacattatttatattatccaataattcgagttacgaattcgagttctaaattatgtatgtagaataaatactt

SEQ ID NO: 14 - DNA, 200 bp, Cucumis sativus
  source 1..200: mol_type = genomic DNA
taaaagtaaacctccttttgaatggacattgtagacttggattttgaatgtataacatatgtattgtcacaccctacccctccagccactacatgcagaaggaggtgtgttgcttagacacccaacgtatacctctctgcgagttgacgagttgaacgcctagtaagtggagcttctcaaaccaatcttcatcatagagt

SEQ ID NO: 15 - DNA, 200 bp, Cucumis sativus
  source 1..200: mol_type = genomic DNA
gtgtatttagaatgacgtacgaaaacatttttcaaaaattcatttttatttaaacatttttaataaaaacctcttaaaatatgttatatacactaaaaatgtttttttattaacttttctcaaaattgataggtaacgacggttgctggagttggttgttgaaagtttgctagtagagtcactgaaggtggtggtcgaag

SEQ ID NO: 16 - DNA, 200 bp, Cucumis sativus
  source 1..200: mol_type = genomic DNA
aatataacatcttcctctaacatccaaccaaatattttagcaatgtatatgctattttaatgtttttaaaaagggagacattgctttcaaaaaagaaaaaggaatttatggtttgagttcattaccttcaatcatgaaccacgctacgtagaataaacgacgtctgagattaagacagagctaagcgagcggttatgttg

SEQ ID NO: 17 - DNA, 200 bp, Cucumis sativus
  source 1..200: mol_type = genomic DNA
aattttaagacataaattccaacaaacaagtttctctaaattttttttccgatagatcccgttgaacatgcatgtgttagattttagaccgttgaattttgcttttttttttaaatttaaatgcttaactagttttttaatttggctaatttatagaaaagtggaaatttcacgtatggaaaaaaaaccaaactatttag

SEQ ID NO: 18 - DNA, 200 bp, Cucumis sativus
  source 1..200: mol_type = genomic DNA
tgtccatgtttcaccaagggaaggtgttaatgtgttttcccaagaagtcggatcacaattgttatgacctcctcatttggtcatttctccaagacgacaaggtaatgtgtctctaacaggtggatttggtttgaatatatttcacaaggatgacattttatgtttttggcaaagggaaagcttgttgatccaagctgacg

SEQ ID NO: 19 - DNA, 200 bp, Cucumis sativus
  source 1..200: mol_type = genomic DNA
acatctacaaaaaatagagatgcaaacaatttaaaaaatttgagaaaaaataaaatcaatttatcaaaaaccaaaactagaaaacaaaatgaatatcaaacggggatgtgtcttgggccttagtttatgtctttgaaggaatacaccttataatctgatgtacaaagaagtccctaattttatagtgagaaagctttctt

SEQ ID NO: 20 - DNA, 2000 bp, Cucumis sativus
  source 1..2000: mol_type = genomic DNA
aaattggaaatgttgatttttatttggagaaagaatattattggtttgaatccatttacttttaaaattaaactttaaatctgaatcttttttagtattttaattattatgatccatatatgtttgttatttagaaaaaaaagtaaaaaattaaaaattaaaaagtccaatttcaatacataaaaaagaaacatgcctaatttaaatttgaggagagtaaaaaagtcaataaaaaaatcgataaaaagggaaaagaaatccataactaaatcgataatgttaaatctaaccaaataaaaacaaatcattggtttttgttgttcattgaacttcagtttggtttcttaattataaaactgatcagtttcgtttggtgatttagttaacctaaacccatacatacaaaaaaattataaaggagtacatagccacattgcaaccattcctttccttgcttcattcatgtttgatctaaaaagattgacaattagatgaaaattgtgtatgctcttttttattgacatttcaattaaaaaaaaaaaaaacaaacatttctctctcaattaaacttgttgaaacccttccttacttcacttatgtacgagtaaataaatcttatcttatcttctctaactctcatctaaaatttgtattcttatattaattctttaacgatataagatgattaagataaggaaaattcaattcatacacatagatttattaatttacaatataaattaagggcgagtgatttgaactacgatcgaacgtctacgcttttaaatgacagttataattgatttttgatactttgatatgtatatatatatatttattaatttgttgtttgtaggcccaacccaaatcaagaatgagagaatgagattcacctaaagtaggtaaggaatctggtttcaaatcctaaatttgtggacctatttcttaaaaacaaaatattaataaaaatatctacctttttccattgcatatacattaatttaatttgtctgacttttcaattttagtgatattagatacttaaaaaaaagttcaaaaatatttattttagtttctataatttaatccctaaacccaataattttggtctttactctacatttctacctaatgccctactttagtaaaaacaatgatgcttaagttaagtcaacaaatgtcctcctaactatttaatatacattgcaatattaagaactataacgtaataacaaaaataatttagaaactagttcatttaaatgacatctaggtttgtggaaggacaaaaatttcatattcaaatatgtggtgtccaaattatactacaataccttttgaaaaggacttatatgatatagataaaaaagaatcaatcataaattttccacctctttgcatggtagatgggcataaacctaactaaaaatttggagacagttaggaaaagagtaatagggagaacgatttggagaagtgtattagaataatatggggagtttgagtgaatatagagttgtatttgtaggataataataataaagagtagaggaatttaaatatatgatttgacatgtatgagtatgcattccgccatccatgtatctaaaaaaaaagtaattcctttttaaaaatttttgtagtggggttttgagggctcccactcccccccgccttcatcacatgcaaacactactactatctactaagtactatccctatatcattaatttacacatttaccctcgcgtggaccccacgctcctactactgaaaattgatcactcagcgcgtggagtcaaaacactatcatcgccgccacatgcgggtttgtctcaatgggcccccccgacatctttttctccaaataataaaatgaaaacccacacgtgtctctctcccattggttattctacgtggacgaatcttattggatgtagtaaaacgacgacatcgtgaacgtcgtcccagtccccagacctcgacacaccatccatctc

SEQ ID NO: 21 - DNA, 20 bp, synthetic construct
  source 1..20: mol_type = other DNA; note = Primer
cgttctcatgttctgccgta

SEQ ID NO: 22 - DNA, 20 bp, synthetic construct
  source 1..20: mol_type = other DNA; note = Primer
ttcgaccaaccggtagaaac

SEQ ID NO: 23 - DNA, 20 bp, synthetic construct
  source 1..20: mol_type = other DNA; note = Primer
taacagccgtggatgtacca

SEQ ID NO: 24 - DNA, 20 bp, synthetic construct
  source 1..20: mol_type = other DNA; note = Primer
atcgcttccagagcattcat

SEQ ID NO: 25 - DNA, 24 bp, synthetic construct
  source 1..24: mol_type = other DNA; note = Primer
caaaacaaggtaaggtgtattgga

SEQ ID NO: 26 - DNA, 20 bp, synthetic construct
  source 1..20: mol_type = other DNA; note = Primer
taaaaggcaggacatgctca

SEQ ID NO: 27 - DNA, 20 bp, synthetic construct
  source 1..20: mol_type = other DNA; note = Primer
cgtggcataaaaccacgaat

SEQ ID NO: 28 - DNA, 22 bp, synthetic construct
  source 1..22: mol_type = other DNA; note = Primer
caaattcaacaaaaccctacca

SEQ ID NO: 29 - DNA, 2000 bp, Cucumis sativus
  source 1..2000: mol_type = genomic DNA
catagcaaatggtatgtgccatctcaccattttcttttcttttttctccatccaccaaaaaatgtgtgccactaatatttattttttccttctattttgcagttagcccgagttcgtatcgtgaaatttggagatactagggttcctatgtattcaagtactttactttattccgttcaacatatgtttttaagttacaatattgtaatatgtacgaaatgttatcaaaaaacactacctatatgacattgtatgtggacactttcataaatttttctaatatagtttataaacttttttttcatgtcttcgatgcatgttacatgcttacctctattttcaaaagttttcgtcccaaagtaattaacatgtttttctcaatggcaaaattacgacacttatatcataagttaccaaacaatcacctacttagtttcttcaacttcatcttctttaaaaaatgtggatatatcttataataatccaagttcttttgcaaaataaaaacaaaactttccaattttgcgttagttttcccgttcactatatctttttatcataatttttttaaaatttttttttgctaattttgtaatttagaaaatagggtgacatgagtactattatcataattttttttttttgtaaacatctctatatttctgtatctaatctagcttgaaattttcaaaatttttgtaatagacccattaatttttaaagtgtacaaaagtatttcttagactcacatttaaattttaagtccaatataatatttataagtttttaactagtatattagtttttaacttttgaacatctaaataagatgtaaatttgatattttgagaatttatcagacaaaaattcaagaatttagtaacatattataatctattaattaaagttaaaaaactatatatagagagacataaatgtaaaagtttatattgcaatcttgtgctctcaatattgaacttctgaatcttgtgaatgaagcagggaagactgaaattaaaccaattctaaacattttatattccataatttaatacgaaattaaaccataatatagaaagaaataaaattgaaaatggaagtgccactttcgttaaaatatcatctcactttattattattattatcataaggaaacatggtatcacatgtggttttcctaaaaaaaaatttaaatccaaatttttaattaaaccgcatgacttatcacgttttcttgtagagtttcttggggttttcttgttctatatatactcataattgaaatgaatagccacaagggaagaaataactaaaattgtgatggcgattgttcttcttattttcttgtttctattcactaattcaaaaggcgaagagataacattcaatgtaaagcaacatctgtccactgttaccaggtaattctcttcatcatcttacctttctcaccccattttgtgtgggtttctttttccttttttctttttgttgattgagagtacgtatgcttgggaatgattttaaagatggatggatgctagcttgtgtttgtttgaaaccttttttaaacattaatcttacatatcaaatggacattttagaaatattcctttattttaaaattagcttaattagcttctgtagatgagaagttgacaagattatgtcaattacatgatcatagcccatgggttctttttcatttataaatttctacttgggtgtaattagcacgtgattttttctacttaaaatgtaattgcacttgtttattatttcaaattttataaaaattttaagttgttcttttataatatatattttttattattcttcatgttgcacatgtaccctatttttataaaatgactttgaaagagatttgtgcaaatttaaatatgtagttaacaaatttcgaacaatacatttgaaatattgagcaaaataatactacttattaattaaaaaaattactatatttataaatattttaagtaatt

SEQ ID NO: 30 - DNA, 2000 bp, Cucumis sativus
  source 1..2000: mol_type = genomic DNA
accctaaaacagggagaaaagccacgatgttattttcttattatttttctctatctcataatgatacagggaacatttatttataggttatagaacccctaataaaaataataaaagataattagggcactataaaatcttaacaaattttcaggctttcaacatacaacaggcctgctaattctaacacacattgttgagaaaatttctccttaaaagccaaggacgcatccttcccatcatcctgagctcatagctttgtgataaccattgtattcccccataattacaaccattcctgcttctttcttaacccaatactcatgcttttccttcaccatcttacttcgaatatgctactcttcgaattacttggtgcctcatctacaacatttcttttcattttaaccataacataagaaatcttagaatgaatccctttactcttaggcttcaaatcaatcccatcttgctttgggatggagtctcttatcattttccaaaaaactatccagcctcttttgctatttcgtgcaggattcatgattgttctcatacctgacctgaaaataacctttttgattatagcttgcctcaagaagcagattttagtggatattgccgactttaatgtagttttaaatttttttatataaataaatttagaaataaaatgtttaattggttgaatgacgaatcctaagagataaaaagatgcccatttattgggattacgaaagatttctccaattttgtaacatgaaaatttaaacttggactgtttaggagctgtaaattttttcgccaatagagagcattgaaaatagataactcaagaatcccagaagctcaggatcttctttcctctgaagtttctttcttcccgaatattcctcaatacagctctgataatggctagctcaaaggtgctctctgtagttgaattgttcttatgaagagagatgtgaataagtgattaccttttcttccaacttgaaaaatccattcagcacgaacccaatggaaaatgactaatctgatagatcaactactaaaatccgtgcttcaaaatatttagttattgaagaacttgaggaagatataagttgctcatatactgtggaaaaccatcctgtttttcattacgccttctctctttgctctccatctctctctacctcctcctgtctggttctgcaaccatcaactttttgcataacttaaccatcgtccaccttcatgactagaccaaccaccattgactagaatgattaccgttgataagaaaacattcttgatagagtttgacccttcttcccctgactctaatgttcaactaacagagtccacttgtaacaaggccttttcattatcgcaccctttggtggatcatggaaactttcaagcccctcctcacggctcctttgaaccaaaaattcttcaaagaacccaaggttgatggccaagtcgtttggataaaaaatgacataaaacaataatggattttctagaaatagttttctttttcatttttttttaagtcaaccgtggaaatagttaagcttgacacaatggggaacaagctgtctactgatttctgcttgagaacaaaggtatggaatgtttttataagattcgctgcattttacagctaaaaagcaactggcaccattaatgggagccaacaactctcatactaggtaatccatcttaatgaaggagccaaaccaaccactaaaccttaaaatagagagtggaaaaccatgggaaagagctaatttattctcccaacctccattaacatactagatctaagatttactgaacgtaaactaattttaagatttatttaaaatacagggactaaatttagacacttggaagtacaaggacaacgattgaattagaccaaaatggtattttagtatagatttcgtatttttgtttagttcccagaatgttcaatgttgtgtaaacaattttaatcccttctatggtca

SEQ ID NO: 31 - DNA, 200 bp, Cucumis sativus
  source 1..200: mol_type = genomic DNA
ttcatcttgttatttacattttgtactccatcaattcttttgaaatttgtttctgacattttggtcattgctcaatattttggttccacaaccaaatctaactcgatctatcttccatacaaaaaaataatatatctttgttttatttaatgtaataaccactcttattctgtgtaagttaaccctattttatataaaaa

SEQ ID NO: 32 - DNA, 200 bp, Cucumis sativus
  source 1..200: mol_type = genomic DNA
gtaaacttgtcccttgcaataaataaatcgttatttcttcatgtttctgtgctgtttaagcagaataattgagcaatatctcacacttcccttatattaaaaaaaagaaaagaaaaaagaaaaaatgatagtggaaaacgcaaacatgtagaaataatgatcgtcgcctctgtctgtttgtgaacaatattttatgtgta

SEQ ID NO: 33 - DNA, 200 bp, Cucumis sativus
  source 1..200: mol_type = genomic DNA
tttattcaaagactagcctatgatagattttgagaaattgtaataatttctcattttctgaaggtgagaaactttccttaaatatgtagtcttaattaatggaatattattctacttattttatgagatcattccttcaaacattggagtaatgaggggtagaaataagacattagtttaaaaataaataaataaatatt

SEQ ID NO: 34 - DNA, 200 bp, Cucumis sativus
  source 1..200: mol_type = genomic DNA
tttattttcaaaattttcgagtttataaaaaaaaagttataaacccaaaacctttttttaaaaaataaagtgggatatctaaatttaaaatttatagaaacggtatacattaaaattgaacaaacttaaaaaatattgatcgatatgtttacttaaaagaacgtatctcaaacaacaaatattatttttgttgtatttat

SEQ ID NO: 35 - DNA, 200 bp, Cucumis sativus
  source 1..200: mol_type = genomic DNA
taaaacactattccattcttaattaacatcttaatgttaattagtaaaatcttaatgttaattagtaaagcgatagtagttcaatcgacctcgttatattaaaaatatttacaaaatagattctaaaatttttattatattttgtaaatattttagttcgatattttattttttaaaatacctatacattgtaattttaa